European Patent Application EP 4 523 694 A1, published March 19, 2025. Title: METHOD AND COMPOSITION BOTH FOR TREATING OR DIAGNOSING INFLAMMATORY BOWEL DISEASE (IBD). Applicant: The University of Tokyo. Application EP EP23803649.5, filed May 12, 2023. The sequence listing filed with the application follows.

SEQUENCE LISTING (137 sequences)

SEQ ID NO: 1 - protein, 5 aa, Mus musculus
SYGIS

SEQ ID NO: 2 - protein, 16 aa, Mus musculus
EIYPRSGNTYYNEKFK

SEQ ID NO: 3 - protein, 8 aa, Mus musculus
FCARLASS

SEQ ID NO: 4 - protein, 11 aa, Mus musculus
KASQDINSYLS

SEQ ID NO: 5 - protein, 7 aa, Mus musculus
RANRLVD

SEQ ID NO: 6 - protein, 9 aa, Mus musculus
LQYDEFPLT

SEQ ID NO: 7 - protein, 144 aa, Mus musculus
MEWIWIFLFILSGTAGVQSQVQLQQSGAELARPGASVKLSCKASGYTFTSYGISWVKQRTGQGLEWIGEIYPRSGNTYYNEKFKGKATLTADKSSSTAYMELRSLTSEDSAVYFCARLASSYYGSSYDWYFDVWGTGTTVTVSS

SEQ ID NO: 8 - protein, 127 aa, Mus musculus
MRTPAQFLGILLLWFPGIKCDIKMTQSPSSMYASLGERVTITCKASQDINSYLSWFQQKPGKSPKTLIYRANRLVDGVPSRFSGSGSGQDYSLTISSLEYEDMGIYYCLQYDEFPLTFGAGTKLELK

SEQ ID NO: 9 - protein, 488 aa, Mus musculus
MEWIWIFLFILSGTAGVQSQVQLQQSGAELARPGASVKLSCKASGYTFTSYGISWVKQRTGQGLEWIGEIYPRSGNTYYNEKFKGKATLTADKSSSTAYMELRSLTSEDSAVYFCARLASSYYGSSYDWYFDVWGTGTTVTVSSESARNPTIYPLTLPRALSSDPVIIGCLIHDYFPSGTMNVTWGKSGKDITTVNFPPALASGGGYTMSSQLTLPAVECPEGESVKCSVQHDSNAVQELDVKCSGPPPPCPPCPPSCHPSLSLQRPALEDLLLGSDASLTCTLNGLRNPEGAVFTWEPSTGKDAVQKKAVQNSCGCYSVSSVLPGCAERWNSGASFKCTVTHPESDTLTGTIAKITVNTFPPQVHLLPPPSEELALNELVSLTCLVRAFNPKEVLVRWLHGNEELSPESYLVFEPLKEPGEGATTYLVTSVLRVSAELWKQGDQYSCMVGHEALPMNFTQKTIDRLSGKPTNVSVSVIMSEGDGICY

SEQ ID NO: 10 - protein, 234 aa, Mus musculus
MRTPAQFLGILLLWFPGIKCDIKMTQSPSSMYASLGERVTITCKASQDINSYLSWFQQKPGKSPKTLIYRANRLVDGVPSRFSGSGSGQDYSLTISSLEYEDMGIYYCLQYDEFPLTFGAGTKLELKRADAAPTVSIFPPSSEQLTSGGASVVCFLNNFYPKDINVKWKIDGSERQNGVLNSWTDQDSKDSTYSMSSTLTLTKDEYERHNSYTCEATHKTSTSPIVKSFNRNEC

SEQ ID NO: 11 - protein, 5 aa, Mus musculus
TFGMG

SEQ ID NO: 12 - protein, 16 aa, Mus musculus
LAHIWWDDDKYYNPAL

SEQ ID NO: 13 - protein, 8 aa, Mus musculus
YYCARIAG

SEQ ID NO: 14 - protein, 11 aa, Mus musculus
SASSSVSYMHW

SEQ ID NO: 15 - protein, 8 aa, Mus musculus
STSNLASG

SEQ ID NO: 16 - protein, 9 aa, Mus musculus
QRSSYPYTF

SEQ ID NO: 17 - protein, 135 aa, Mus musculus
MGRLTSSFLLLIVPAYVLSQVTLKESGPGILQPSQTLSLTCSFSGFSLSTFGMGVGWIRQPSGKGLEWLAHIWWDDDKYYNPALKSRLTISKDTSKNQVFLKIANVDTADTATYYCARIAGFDYWGQGTTLTVSS

SEQ ID NO: 18 - protein, 128 aa, Mus musculus
MHFQVQIFSFLLISASVIMSRGQIVLTQSPAIMSASPGEKVTITCSASSSVSYMHWFQQKPGTSPKLWIYSTSNLASGVPARFSGSGSGTSYSLTISRMEAEDAATYYCQQRSSYPYTFGGGTKLEIK

SEQ ID NO: 19 - protein, 479 aa, Mus musculus
MGRLTSSFLLLIVPAYVLSQVTLKESGPGILQPSQTLSLTCSFSGFSLSTFGMGVGWIRQPSGKGLEWLAHIWWDDDKYYNPALKSRLTISKDTSKNQVFLKIANVDTADTATYYCARIAGFDYWGQGTTLTVSSESARNPTIYPLTLPRALSSDPVIIGCLIHDYFPSGTMNVTWGKSGKDITTVNFPPALASGGGYTMSSQLTLPAVECPEGESVKCSVQHDSNAVQELDVKCSGPPPPCPPCPPSCHPSLSLQRPALEDLLLGSDASLTCTLNGLRNPEGAVFTWEPSTGKDAVQKKAVQNSCGCYSVSSVLPGCAERWNSGASFKCTVTHPESDTLTGTIAKITVNTFPPQVHLLPPPSEELALNELVSLTCLVRAFNPKEVLVRWLHGNEELSPESYLVFEPLKEPGEGATTYLVTSVLRVSAELWKQGDQYSCMVGHEALPMNFTQKTIDRLSGKPTNVSVSVIMSEGDGICY

SEQ ID NO: 20 - protein, 235 aa, Mus musculus
MHFQVQIFSFLLISASVIMSRGQIVLTQSPAIMSASPGEKVTITCSASSSVSYMHWFQQKPGTSPKLWIYSTSNLASGVPARFSGSGSGTSYSLTISRMEAEDAATYYCQQRSSYPYTFGGGTKLEIKRADAAPTVSIFPPSSEQLTSGGASVVCFLNNFYPKDINVKWKIDGSERQNGVLNSWTDQDSKDSTYSMSSTLTLTKDEYERHNSYTCEATHKTSTSPIVKSFNRNEC

SEQ ID NO: 21 - protein, 5 aa, Mus musculus
SYNIH

SEQ ID NO: 22 - protein, 16 aa, Mus musculus
AIYSGNGATSHNQKFK

SEQ ID NO: 23 - protein, 8 aa, Mus musculus
FCTRVGLR

SEQ ID NO: 24 - protein, 11 aa, Mus musculus
KASQSVGTSVA

SEQ ID NO: 25 - protein, 7 aa, Mus musculus
SASYRYS

SEQ ID NO: 26 - protein, 9 aa, Mus musculus
QQYNNYPYT

SEQ ID NO: 27 - protein, 137 aa, Mus musculus
MGFSRIFLFLLSVTTGVHSQAYLQQSGAELVRPGASVRMSCKASDYTFTSYNIHWVKQTPRQGLEWIGAIYSGNGATSHNQKFKGRATLTVDKSSSTAYMQLSSLTSEDSAVYFCTRVGLRSPFDFWGQGTTLTVSS

SEQ ID NO: 28 - protein, 127 aa, Mus musculus
MESQTQVFVYMLLWLSGVDGDIVMTQSLKFMSTSGGDRVSVTCKASQSVGTSVAWYQQKPGQSPKPLIYSASYRYSGVPDRFTGSGSGTDFSLTISNVQSEDLAEYFCQQYNNYPYTFGGGTKLEIK

SEQ ID NO: 29 - protein, 481 aa, Mus musculus
MGFSRIFLFLLSVTTGVHSQAYLQQSGAELVRPGASVRMSCKASDYTFTSYNIHWVKQTPRQGLEWIGAIYSGNGATSHNQKFKGRATLTVDKSSSTAYMQLSSLTSEDSAVYFCTRVGLRSPFDFWGQGTTLTVSSESARNPTIYPLTLPRALSSDPVIIGCLIHDYFPSGTMNVTWGKSGKDITTVNFPPALASGGGYTMSSQLTLPAVECPEGESVKCSVQHDSNAVQELDVKCSGPPPPCPPCPPSCHPSLSLQRPALEDLLLGSDASLTCTLNGLRNPEGAVFTWEPSTGKDAVQKKAVQNSCGCYSVSSVLPGCAERWNSGASFKCTVTHPESDTLTGTIAKITVNTFPPQVHLLPPPSEELALNELVSLTCLVRAFNPKEVLVRWLHGNEELSPESYLVFEPLKEPGEGATTYLVTSVLRVSAELWKQGDQYSCMVGHEALPMNFTQKTIDRLSGKPTNVSVSVIMSEGDGICY

SEQ ID NO: 30 - protein, 234 aa, Mus musculus
MESQTQVFVYMLLWLSGVDGDIVMTQSLKFMSTSGGDRVSVTCKASQSVGTSVAWYQQKPGQSPKPLIYSASYRYSGVPDRFTGSGSGTDFSLTISNVQSEDLAEYFCQQYNNYPYTFGGGTKLEIKRADAAPTVSIFPPSSEQLTSGGASVVCFLNNFYPKDINVKWKIDGSERQNGVLNSWTDQDSKDSTYSMSSTLTLTKDEYERHNSYTCEATHKTSTSPIVKSFNRNEC

SEQ ID NO: 31 - protein, 5 aa, Mus musculus
DYYIH

SEQ ID NO: 32 - protein, 16 aa, Mus musculus
RIDPENDETTYAPKFQ

SEQ ID NO: 33 - protein, 8 aa, Mus musculus
YCARSTVL

SEQ ID NO: 34 - protein, 11 aa, Mus musculus
RASQSIVHTNG

SEQ ID NO: 35 - protein, 7 aa, Mus musculus
KLLIYKV

SEQ ID NO: 36 - protein, 9 aa, Mus musculus
GVYYCFQGS

SEQ ID NO: 37 - protein, 134 aa, Mus musculus
MKCSWIIFFLMAVVTGVNSEVQLQQSGSELVKSGASVKLSCTVSGFNFTDYYIHWVRQRTEQGLEWIGRIDPENDETTYAPKFQGKATMTADTSSNTAYLQLTSLTSEDTAVYYCARSTVLDYWGHGTTLTVSS

SEQ ID NO: 38 - protein, 131 aa, Mus musculus
MKLPVRLLVLMFWIPGFSSDVLMTQTPLSLPVSLGDQASISCRASQSIVHTNGNTYLEWYLQKPGQSPKLLIYKVSNRFSGVPDRFSGSGSGTDFILKISRVEAEDLGVYYCFQGSHVPPTFGGGTKLEVK

SEQ ID NO: 39 - protein, 478 aa, Mus musculus
MKCSWIIFFLMAVVTGVNSEVQLQQSGSELVKSGASVKLSCTVSGFNFTDYYIHWVRQRTEQGLEWIGRIDPENDETTYAPKFQGKATMTADTSSNTAYLQLTSLTSEDTAVYYCARSTVLDYWGHGTTLTVSSESARNPTIYPLTLPRALSSDPVIIGCLIHDYFPSGTMNVTWGKSGKDITTVNFPPALASGGGYTMSSQLTLPAVECPEGESVKCSVQHDSNAVQELDVKCSGPPPPCPPCPPSCHPSLSLQRPALEDLLLGSDASLTCTLNGLRNPEGAVFTWEPSTGKDAVQKKAVQNSCGCYSVSSVLPGCAERWNSGASFKCTVTHPESDTLTGTIAKITVNTFPPQVHLLPPPSEELALNELVSLTCLVRAFNPKEVLVRWLHGNEELSPESYLVFEPLKEPGEGATTYLVTSVLRVSAELWKQGDQYSCMVGHEALPMNFTQKTIDRLSGKPTNVSVSVIMSEGDGICY

SEQ ID NO: 40 - protein, 238 aa, Mus musculus
MKLPVRLLVLMFWIPGFSSDVLMTQTPLSLPVSLGDQASISCRASQSIVHTNGNTYLEWYLQKPGQSPKLLIYKVSNRFSGVPDRFSGSGSGTDFILKISRVEAEDLGVYYCFQGSHVPPTFGGGTKLEVKRADAAPTVSIFPPSSEQLTSGGASVVCFLNNFYPKDINVKWKIDGSERQNGVLNSWTDQDSKDSTYSMSSTLTLTKDEYERHNSYTCEATHKTSTSPIVKSFNRNEC

SEQ ID NO: 41 - protein, 5 aa, synthetic construct
NYYIH

SEQ ID NO: 42 - protein, 16 aa, synthetic construct
RIDPENNETTYAPKFQ

SEQ ID NO: 43 - protein, 16 aa, synthetic construct
RIDPENDQTTYAPKFQ

SEQ ID NO: 44 - protein, 16 aa, synthetic construct
RIDPENNQTTYAPKFQ

SEQ ID NO: 45 - protein, 134 aa, synthetic construct
MKCSWIIFFLMAVVTGVNSEVQLQQSGSELVKSGASVKLSCTVSGFNFTNYYIHWVRQRTEQGLEWIGRIDPENDETTYAPKFQGKATMTADTSSNTAYLQLTSLTSEDTAVYYCARSTVLDYWGHGTTLTVSS

SEQ ID NO: 46 - protein, 134 aa, synthetic construct
MKCSWIIFFLMAVVTGVNSEVQLQQSGSELVKSGASVKLSCTVSGFNFTDYYIHWVRQRTEQGLEWIGRIDPENNETTYAPKFQGKATMTADTSSNTAYLQLTSLTSEDTAVYYCARSTVLDYWGHGTTLTVSS

SEQ ID NO: 47 - protein, 134 aa, synthetic construct
MKCSWIIFFLMAVVTGVNSEVQLQQSGSELVKSGASVKLSCTVSGFNFTDYYIHWVRQRTEQGLEWIGRIDPENDQTTYAPKFQGKATMTADTSSNTAYLQLTSLTSEDTAVYYCARSTVLDYWGHGTTLTVSS

SEQ ID NO: 48 - protein, 134 aa, synthetic construct
MKCSWIIFFLMAVVTGVNSEVQLQQSGSELVKSGASVKLSCTVSGFNFTNYYIHWVRQRTEQGLEWIGRIDPENNETTYAPKFQGKATMTADTSSNTAYLQLTSLTSEDTAVYYCARSTVLDYWGHGTTLTVSS

SEQ ID NO: 49 - protein, 134 aa, synthetic construct
MKCSWIIFFLMAVVTGVNSEVQLQQSGSELVKSGASVKLSCTVSGFNFTNYYIHWVRQRTEQGLEWIGRIDPENDQTTYAPKFQGKATMTADTSSNTAYLQLTSLTSEDTAVYYCARSTVLDYWGHGTTLTVSS

SEQ ID NO: 50 - protein, 134 aa, synthetic construct
MKCSWIIFFLMAVVTGVNSEVQLQQSGSELVKSGASVKLSCTVSGFNFTDYYIHWVRQRTEQGLEWIGRIDPENNQTTYAPKFQGKATMTADTSSNTAYLQLTSLTSEDTAVYYCARSTVLDYWGHGTTLTVSS

SEQ ID NO: 51 - protein, 134 aa, synthetic construct
MKCSWIIFFLMAVVTGVNSEVQLQQSGSELVKSGASVKLSCTVSGFNFTNYYIHWVRQRTEQGLEWIGRIDPENNQTTYAPKFQGKATMTADTSSNTAYLQLTSLTSEDTAVYYCARSTVLDYWGHGTTLTVSS

SEQ ID NO: 52 - protein, 11 aa, synthetic construct
RSSQSIVHTNG

SEQ ID NO: 53 - protein, 13 aa, synthetic construct
SPASLSVSLGDRA

SEQ ID NO: 54 - protein, 13 aa, synthetic construct
SPASLSVSLGDRV

SEQ ID NO: 55 - protein, 13 aa, synthetic construct
SPASMSVSLGDRA

SEQ ID NO: 56 - protein, 13 aa, synthetic construct
TPLSLPVSLGDQA

SEQ ID NO: 57 - protein, 131 aa, synthetic construct
MKLPVRLLVLMFWIPGFSSDVLMTQSPASLSVSLGDRATISCRASQSIVHTNGNTYLEWYLQKPGQSPKLLIYKVSNRFSGVPDRFSGSGSGTDFILKISRVEAEDLGVYYCFQGSHVPPTFGGGTKLEVK

SEQ ID NO: 58 - protein, 131 aa, synthetic construct
MKLPVRLLVLMFWIPGFSSDVLMTQSPASLSVSLGDRVTISCRASQSIVHTNGNTYLEWYLQKPGQSPKLLIYKVSNRFSGVPDRFSGSGSGTDFILKISRVEAEDLGVYYCFQGSHVPPTFGGGTKLEVK

SEQ ID NO: 59 - protein, 131 aa, synthetic construct
MKLPVRLLVLMFWIPGFSSDVLMTQSPASLSVSLGDRVTISCRSSQSIVHTNGNTYLEWYLQKPGQSPKLLIYKVSNRFSGVPDRFSGSGSGTDFILKISRVEAEDLGVYYCFQGSHVPPTFGGGTKLEVK

SEQ ID NO: 60 - protein, 131 aa, synthetic construct
MKLPVRLLVLMFWIPGFSSDVLMTQSPASMSVSLGDRATISCRSSQSIVHTNGNTYLEWYLQKPGQSPKLLIYKVSNRFSGVPDRFSGSGSGTDFILKISRVEAEDLGVYYCFQGSHVPPTFGGGTKLEVK

SEQ ID NO: 61 - protein, 131 aa, synthetic construct
MKLPVRLLVLMFWIPGFSSDVLMTQSPASLSVSLGDRATISCRSSQSIVHTNGNTYLEWYLQKPGQSPKLLIYKVSNRFSGVPDRFSGSGSGTDFILKISRVEAEDLGVYYCFQGSHVPPTFGGGTKLEVK

SEQ ID NO: 62 - protein, 5 aa, synthetic construct
XYYIH

SEQ ID NO: 63 - protein, 16 aa, synthetic construct
RIDPENXXTTYAPKFQ

SEQ ID NO: 64 - protein, 11 aa, synthetic construct
RXSQSIVHTNG

SEQ ID NO: 65 - DNA, 1467 bp, Mus musculus
  source 1..1467: mol_type = other DNA
atggaatggatctggatctttctcttcatcctgtcaggaactgcaggtgtccaatcccaggttcagctgcagcagtctggagctgagctggcgaggcctggggcttcagtgaagctgtcctgcaaggcttctggctacaccttcacaagctatggtataagctgggtgaagcagagaactggacagggccttgagtggattggagagatttatcctagaagtggtaatacttactacaatgagaagttcaagggcaaggccacactgactgcagacaaatcctccagcacagcgtacatggagctccgcagcctgacatctgaggactctgcggtctatttctgtgcaagattggcatcgagctactacggtagtagctacgactggtacttcgatgtctggggcacagggaccacggtcaccgtctcctcagagtctgcgagaaatcccaccatctacccactgacactcccacgagctctgtcaagtgacccagtgataatcggctgcctgattcacgattacttcccttccggcacgatgaatgtgacctggggaaagagtgggaaggatataaccaccgtaaacttcccacctgccctggcctctgggggagggtacaccatgagcagccagttgaccctgccagctgtcgagtgcccagaaggagaatccgtgaaatgttccgtgcaacatgactctaacgccgtccaagaattggatgtgaagtgctctggtcctcctcctccttgtcctccttgtcctccttcctgccatcccagcctgtcactgcagcggccagctcttgaggacctgctcctgggttcagatgccagcctcacatgtactctgaatggcctgagaaatcctgagggagctgtcttcacctgggagccctccactgggaaggatgcagtgcagaagaaagctgtgcagaattcctgcggctgctacagtgtgtccagcgtcctgcctggctgtgctgagcgctggaacagtggcgcatcattcaagtgcacagttacccatcctgagtctgacaccttaactggcacaattgccaaaatcacagtgaacaccttcccaccccaggtccacctgctaccgccgccgtcggaggagctggccctgaatgagctcgtgtccctgacatgcctggtgcgagctttcaaccctaaagaagtgctggtgcgatggctgcatggaaatgaggagctgtccccagaaagctacctagtgtttgagcccctaaaggagccaggcgagggagccaccacctacctggtgacaagcgtgttgcgtgtatcagctgaactctggaaacagggtgaccagtactcctgcatggtgggccacgaggccttgcccatgaacttcacccagaagaccatcgaccgtctgtcgggtaaacccaccaatgtcagcgtgtctgtgatcatgtcagagggagatggcatctgctactga

SEQ ID NO: 66 - DNA, 705 bp, Mus musculus
  source 1..705: mol_type = other DNA
atgaggacccctgctcagtttcttggaatcttgttgctctggtttccaggtatcaaatgtgacatcaagatgacccagtctccatcttccatgtatgcatctctaggagagagagtcactatcacttgcaaggcgagtcaggacattaatagctatttaagctggttccagcagaaaccagggaaatctcctaagaccctgatctatcgtgcaaacagattggtagatggggtcccatcaaggttcagtggcagtggatctgggcaagattattctctcaccatcagcagcctggagtatgaagatatgggaatttattattgtctacagtatgatgagtttccgctcacgttcggtgctgggaccaagctggagctgaaacgggctgatgctgcaccaactgtatccatcttcccaccatccagtgagcagttaacatctggaggtgcctcagtcgtgtgcttcttgaacaacttctaccccaaagacatcaatgtcaagtggaagattgatggcagtgaacgacaaaatggcgtcctgaacagttggactgatcaggacagcaaagacagcacctacagcatgagcagcaccctcacgttgaccaaggacgagtatgaacgacataacagctatacctgtgaggccactcacaagacatcaacttcacccattgtcaagagcttcaacaggaatgagtgttga

SEQ ID NO: 67 - DNA, 1440 bp, Mus musculus
  source 1..1440: mol_type = other DNA
atgggcaggcttacttcttcattcctgttactgattgtccctgcatatgtcctgtcccaggttactctgaaagagtctggccctgggatattgcagccctcccagaccctcagtctgacttgttctttctctgggttttcactgagcacttttggtatgggtgtaggctggattcgtcagccttcagggaagggtctggagtggctggcacacatttggtgggatgatgataagtactataacccagccctgaagagtcggctcacaatctccaaggatacctccaaaaaccaggtattcctcaagatcgccaatgtggacactgcagatactgccacatactactgtgctcgaatagctgggtttgactactggggccaaggcaccactctcacagtctcctcagagtctgcgagaaatcccaccatctacccactgacactcccacgagctctgtcaagtgacccagtgataatcggctgcctgattcacgattacttcccttccggcacgatgaatgtgacctggggaaagagtgggaaggatataaccaccgtaaacttcccacctgccctggcctctgggggagggtacaccatgagcagccagttgaccctgccagctgtcgagtgcccagaaggagaatccgtgaaatgttccgtgcaacatgactctaacgccgtccaagaattggatgtgaagtgctctggtcctcctcctccttgtcctccttgtcctccttcctgccatcccagcctgtcactgcagcggccagctcttgaggacctgctcctgggttcagatgccagcctcacatgtactctgaatggcctgagaaatcctgagggagctgtcttcacctgggagccctccactgggaaggatgcagtgcagaagaaagctgtgcagaattcctgcggctgctacagtgtgtccagcgtcctgcctggctgtgctgagcgctggaacagtggcgcatcattcaagtgcacagttacccatcctgagtctgacaccttaactggcacaattgccaaaatcacagtgaacaccttcccaccccaggtccacctgctaccgccgccgtcggaggagctggccctgaatgagctcgtgtccctgacatgcctggtgcgagctttcaaccctaaagaagtgctggtgcgatggctgcatggaaatgaggagctgtccccagaaagctacctagtgtttgagcccctaaaggagccaggcgagggagccaccacctacctggtgacaagcgtgttgcgtgtatcagctgaactctggaaacagggtgaccagtactcctgcatggtgggccacgaggccttgcccatgaacttcacccagaagaccatcgaccgtctgtcgggtaaacccaccaatgtcagcgtgtctgtgatcatgtcagagggagatggcatctgctactga

SEQ ID NO: 68 - DNA, 708 bp, Mus musculus
  source 1..708: mol_type = other DNA
atgcattttcaagtgcagattttcagcttcctgctaatcagtgcctcagtcataatgtccagaggacaaattgttctcacccagtctccagcaatcatgtctgcatctccaggggagaaggtcaccataacctgcagtgccagctcaagtgtaagttacatgcactggttccagcagaagccaggcacttctcccaaactctggatttatagcacatccaacctggcttctggagtccctgctcgcttcagtggcagtggatctgggacctcttactctctcacaatcagccgaatggaggctgaagatgctgccacttattactgccagcaaaggagtagttacccgtacacgttcggaggggggaccaagctggaaataaaacgggctgatgctgcaccaactgtatccatcttcccaccatccagtgagcagttaacatctggaggtgcctcagtcgtgtgcttcttgaacaacttctaccccaaagacatcaatgtcaagtggaagattgatggcagtgaacgacaaaatggcgtcctgaacagttggactgatcaggacagcaaagacagcacctacagcatgagcagcaccctcacgttgaccaaggacgagtatgaacgacataacagctatacctgtgaggccactcacaagacatcaacttcacccattgtcaagagcttcaacaggaatgagtgttga

SEQ ID NO: 69 - DNA, 1446 bp, Mus musculus
  source 1..1446: mol_type = other DNA
atgggattcagcaggatctttctcttcctcctgtcagtaactacaggtgtccactcccaggcttatctacagcagtctggggctgagctggtgaggcctggggcctcagtgaggatgtcctgcaaggcttctgactacacatttaccagttacaatatccactgggtaaagcagacacctagacagggcctggaatggattggagctatttattcaggaaatggtgctacttcccacaatcagaagttcaagggcagggccacactgactgtagacaaatcctccagcacagcctacatgcaactcagcagcctgacatctgaagactctgcggtctatttctgtacaagagtgggactccggtccccttttgacttctggggccaaggcaccactctcacagtctcctcagagtctgcgagaaatcccaccatctacccactgacactcccacgagctctgtcaagtgacccagtgataatcggctgcctgattcacgattacttcccttccggcacgatgaatgtgacctggggaaagagtgggaaggatataaccaccgtaaacttcccacctgccctggcctctgggggagggtacaccatgagcagccagttgaccctgccagctgtcgagtgcccagaaggagaatccgtgaaatgttccgtgcaacatgactctaacgccgtccaagaattggatgtgaagtgctctggtcctcctcctccttgtcctccttgtcctccttcctgccatcccagcctgtcactgcagcggccagctcttgaggacctgctcctgggttcagatgccagcctcacatgtactctgaatggcctgagaaatcctgagggagctgtcttcacctgggagccctccactgggaaggatgcagtgcagaagaaagctgtgcagaattcctgcggctgctacagtgtgtccagcgtcctgcctggctgtgctgagcgctggaacagtggcgcatcattcaagtgcacagttacccatcctgagtctgacaccttaactggcacaattgccaaaatcacagtgaacaccttcccaccccaggtccacctgctaccgccgccgtcggaggagctggccctgaatgagctcgtgtccctgacatgcctggtgcgagctttcaaccctaaagaagtgctggtgcgatggctgcatggaaatgaggagctgtccccagaaagctacctagtgtttgagcccctaaaggagccaggcgagggagccaccacctacctggtgacaagcgtgttgcgtgtatcagctgaactctggaaacagggtgaccagtactcctgcatggtgggccacgaggccttgcccatgaacttcacccagaagaccatcgaccgtctgtcgggtaaacccaccaatgtcagcgtgtctgtgatcatgtcagagggagatggcatctgctactga

SEQ ID NO: 70 - DNA, 705 bp, Mus musculus
  source 1..705: mol_type = other DNA
atggagtcacagactcaggtctttgtatacatgttgctgtggttgtctggtgttgatggagacattgtgatgacccagtctctaaaattcatgtccacatcgggaggagacagggtcagcgtcacctgcaaggccagtcagagtgtgggtacaagtgtagcctggtatcagcagaaaccaggacaatctcctaaaccactgatttattcggcatcttatcggtacagtggagtccctgatcgcttcacaggcagtggatctgggacagatttcagtctcaccatcagcaatgtgcagtctgaagacttggcagaatatttctgtcagcaatataacaactatccgtacacgttcggaggggggaccaagctggagataaaacgggctgatgctgcaccaactgtatccatcttcccaccatccagtgagcagttaacatctggaggtgcctcagtcgtgtgcttcttgaacaacttctaccccaaagacatcaatgtcaagtggaagattgatggcagtgaacgacaaaatggcgtcctgaacagttggactgatcaggacagcaaagacagcacctacagcatgagcagcaccctcacgttgaccaaggacgagtatgaacgacataacagctatacctgtgaggccactcacaagacatcaacttcacccattgtcaagagcttcaacaggaatgagtgttga

SEQ ID NO: 71 - DNA, 1437 bp, Mus musculus
  source 1..1437: mol_type = other DNA
atgaaatgcagctggatcatcttcttcctgatggcagtggttacaggggtcaattcagaggttcagctgcagcagtctgggtcagagcttgtgaagtctggggcctcagtcaagttgtcctgcacagtttctgggttcaactttacagactactatatacactgggtgaggcagaggactgaacagggcctggaatggattggaaggattgatcctgagaatgatgaaactacatatgccccgaaattccagggcaaggccactatgacagcagacacatcttccaacacagcctacctgcagctcaccagcctgacatctgaagacactgccgtctattactgtgctagatctacggtccttgactactggggccacggcaccactctcacagtctcctcagagtctgcgagaaatcccaccatctacccactgacactcccacgagctctgtcaagtgacccagtgataatcggctgcctgattcacgattacttcccttccggcacgatgaatgtgacctggggaaagagtgggaaggatataaccaccgtaaacttcccacctgccctggcctctgggggagggtacaccatgagcagccagttgaccctgccagctgtcgagtgcccagaaggagaatccgtgaaatgttccgtgcaacatgactctaacgccgtccaagaattggatgtgaagtgctctggtcctcctcctccttgtcctccttgtcctccttcctgccatcccagcctgtcactgcagcggccagctcttgaggacctgctcctgggttcagatgccagcctcacatgtactctgaatggcctgagaaatcctgagggagctgtcttcacctgggagccctccactgggaaggatgcagtgcagaagaaagctgtgcagaattcctgcggctgctacagtgtgtccagcgtcctgcctggctgtgctgagcgctggaacagtggcgcatcattcaagtgcacagttacccatcctgagtctgacaccttaactggcacaattgccaaaatcacagtgaacaccttcccaccccaggtccacctgctaccgccgccgtcggaggagctggccctgaatgagctcgtgtccctgacatgcctggtgcgagctttcaaccctaaagaagtgctggtgcgatggctgcatggaaatgaggagctgtccccagaaagctacctagtgtttgagcccctaaaggagccaggcgagggagccaccacctacctggtgacaagcgtgttgcgtgtatcagctgaactctggaaacagggtgaccagtactcctgcatggtgggccacgaggccttgcccatgaacttcacccagaagaccatcgaccgtctgtcgggtaaacccaccaatgtcagcgtgtctgtgatcatgtcagagggagatggcatctgctactga

SEQ ID NO: 72 - DNA, 717 bp, Mus musculus
  source 1..717: mol_type = other DNA
atgaagttgcctgttaggctgttggtgctgatgttctggattcctggattcagcagtgatgttttgatgacccaaactccactctccctgcctgtcagtcttggagatcaagcctccatctcttgtagagctagtcagagcattgtacacactaatgggaacacctatttagaatggtacctgcagaaaccaggccagtctccaaagctcctgatctacaaagtttccaaccgattttctggggtcccagacaggttcagtggcagtggatctgggacagatttcatactcaagatcagcagagtggaggctgaggatctgggagtttattactgctttcaaggttcacatgttcctccgacgttcggtggaggcaccaagctggaagtcaaacgggctgatgctgcaccaactgtatccatcttcccaccatccagtgagcagttaacatctggaggtgcctcagtcgtgtgcttcttgaacaacttctaccccaaagacatcaatgtcaagtggaagattgatggcagtgaacgacaaaatggcgtcctgaacagttggactgatcaggacagcaaagacagcacctacagcatgagcagcaccctcacgttgaccaaggacgagtatgaacgacataacagctatacctgtgaggccactcacaagacatcaacttcacccattgtcaagagcttcaacaggaatgagtgttag

SEQ ID NO: 73 - DNA, 1374 bp, Mus musculus
  source 1..1374: mol_type = other DNA
atgaaatgcagctggatcatcttcttcctgatggcagtggttacaggggtcaattcagaggttcagctgcagcagtctgggtcagagcttgtgaagtctggggcctcagtcaagttgtcctgcacagtttctgggttcaactttacagactactatatacactgggtgaggcagaggactgaacagggcctggaatggattggaaggattgatcctgagaatgatgaaactacatatgccccgaaattccagggcaaggccactatgacagcagacacatcttccaacacagcctacctgcagctcaccagcctgacatctgaagacactgccgtctattactgtgctagatctacggtccttgactactggggccacggcaccactctcacagtctcctcaaaaacgacacccccatctgtctatccactggcccctggatctgctgcccaaactaactccatggtgaccctgggatgcctggtcaagggctatttccctgagccagtgacagtgacctggaactctggatccctgtccagcggtgtgcacaccttcccagctgtcctgcagtctgacctctacactctgagcagctcagtgactgtcccctccagcacctggcccagcgagaccgtcacctgcaacgttgcccacccggccagcagcaccaaggtggacaagaaaattgtgcccagggattgtggttgtaagccttgcatatgtacagtcccagaagtatcatctgtcttcatcttccccccaaagcccaaggatgtgctcaccattactctgactcctaaggtcacgtgtgttgtggtagacatcagcaaggatgatcccgaggtccagttcagctggtttgtagatgatgtggaggtgcacacagctcagacgcaaccccgggaggagcagttcaacagcactttccgctcagtcagtgaacttcccatcatgcaccaggactggctcaatggcaaggagttcaaatgcagggtcaacagtgcagctttccctgcccccatcgagaaaaccatctccaaaaccaaaggcagaccgaaggctccacaggtgtacaccattccacctcccaaggagcagatggccaaggataaagtcagtctgacctgcatgataacagacttcttccctgaagacattactgtggagtggcagtggaatgggcagccagcggagaactacaagaacactcagcccatcatggacacagatggctcttacttcgtctacagcaagctcaatgtgcagaagagcaactgggaggcaggaaatactttcacctgctctgtgttacatgagggcctgcacaaccaccatactgagaagagcctctcccactctcctggtaaataa

SEQ ID NO: 74 - DNA, 1407 bp, synthetic construct
  source 1..1407: mol_type = other DNA
atgaaatgcagctggatcatcttcttcctgatggcagtggttacaggggtcaattcagaggttcagctgcagcagtctgggtcagagcttgtgaagtctggggcctcagtcaagttgtcctgcacagtttctgggttcaactttacagactactatatacactgggtgaggcagaggactgaacagggcctggaatggattggaaggattgatcctgagaatgatgaaactacatatgccccgaaattccagggcaaggccactatgacagcagacacatcttccaacacagcctacctgcagctcaccagcctgacatctgaagacactgccgtctattactgtgctagatctacggtccttgactactggggccacggcaccactctcacagtctcctcagcatccccgactagttccaccaagggcccatcggtcttccccctggcaccctcctccaagagcacctctgggggcacagcggccctgggctgcctggtcaaggactacttccccgaaccggtgacggtgtcgtggaactcaggcgccctgaccagcggcgtgcacaccttcccggctgtcctacagtcctcaggactctactccctcagcagcgtggtgaccgtgccctccagcagcttgggcacccagacctacatctgcaacgtgaatcacaagcccagcaacaccaaggtggacaagaaagttgagcccaaatcttgtgacaaaactcacacatgcccaccgtgcccagcacctgaactcctggggggaccgtcagtcttcctcttccccccaaaacccaaggacaccctcatgatctcccggacccctgaggtcacatgcgtggtggtggacgtgagccacgaagaccctgaggtcaagttcaactggtacgtggacggcgtggaggtgcataatgccaagacaaagccgcgggaggagcagtacaacagcacgtaccgtgtggtcagcgtcctcaccgtcctgcaccaggactggctgaatggcaaggagtacaagtgcaaggtctccaacaaagccctcccagcccctatcgagaaaaccatctccaaagccaaagggcagccccgagaaccacaggtgtacaccctgcccccatcccgggatgagctgaccaagaaccaggtcagcctgacctgcctggtcaaaggcttctatcccagcgacatcgccgtggagtgggagagcaatgggcagccggagaacaactacaagaccacgcctcccgtgctggactccgacggctccttcttcctctacagcaagctcaccgtggacaagagcaggtggcagcaggggaacgtcttctcatgctccgtgatgcatgagggtctgcacaaccactacacgcagaagagcctctccctgtctccgggtaaatga

SEQ ID NO: 75 - DNA, 723 bp, synthetic construct
  source 1..723: mol_type = other DNA
atggacatgaagttgcctgttaggctgttggtgctgatgttctggattcctggattcagcagtgatgttttgatgacccaaactccactctccctgcctgtcagtcttggagatcaagcctccatctcttgtagagctagtcagagcattgtacacactaatgggaacacctatttagaatggtacctgcagaaaccaggccagtctccaaagctcctgatctacaaagtttccaaccgattttctggggtcccagacaggttcagtggcagtggatctgggacagatttcatactcaagatcagcagagtggaggctgaggatctgggagtttattactgctttcaaggttcacatgttcctccgacgttcggtggaggcaccaagctggaagtcaaacgggctgatgctgcaccaactgtatccatcttcccaccatccagtgagcagttaacatctggaggtgcctctgttgtgtgcctgctgaataacttctatcctcgagaggccaaagtacagtggaaggtggataacgccctccaatcgggtaactcccaggagagtgtcacagagcaggacagcaaggacagcacctacagcctcagcagcaccctgacgctgagcaaagcagactacgagaaacacaaagtctacgcctgcgaagtcacccatcagggcctgagctcgcccgtcacaaagagcttcaacaggggagagtgttag

SEQ ID NO: 76 - protein, 457 aa, Mus musculus
MKCSWIIFFLMAVVTGVNSEVQLQQSGSELVKSGASVKLSCTVSGFNFTDYYIHWVRQRTEQGLEWIGRIDPENDETTYAPKFQGKATMTADTSSNTAYLQLTSLTSEDTAVYYCARSTVLDYWGHGTTLTVSSKTTPPSVYPLAPGSAAQTNSMVTLGCLVKGYFPEPVTVTWNSGSLSSGVHTFPAVLQSDLYTLSSSVTVPSSTWPSETVTCNVAHPASSTKVDKKIVPRDCGCKPCICTVPEVSSVFIFPPKPKDVLTITLTPKVTCVVVDISKDDPEVQFSWFVDDVEVHTAQTQPREEQFNSTFRSVSELPIMHQDWLNGKEFKCRVNSAAFPAPIEKTISKTKGRPKAPQVYTIPPPKEQMAKDKVSLTCMITDFFPEDITVEWQWNGQPAENYKNTQPIMDTDGSYFVYSKLNVQKSNWEAGNTFTCSVLHEGLHNHHTEKSLSHSPGK

SEQ ID NO: 77 - protein, 468 aa, synthetic construct
MKCSWIIFFLMAVVTGVNSEVQLQQSGSELVKSGASVKLSCTVSGFNFTDYYIHWVRQRTEQGLEWIGRIDPENDETTYAPKFQGKATMTADTSSNTAYLQLTSLTSEDTAVYYCARSTVLDYWGHGTTLTVSSASPTSSTKGPSVFPLAPSSKSTSGGTAALGCLVKDYFPEPVTVSWNSGALTSGVHTFPAVLQSSGLYSLSSVVTVPSSSLGTQTYICNVNHKPSNTKVDKKVEPKSCDKTHTCPPCPAPELLGGPSVFLFPPKPKDTLMISRTPEVTCVVVDVSHEDPEVKFNWYVDGVEVHNAKTKPREEQYNSTYRVVSVLTVLHQDWLNGKEYKCKVSNKALPAPIEKTISKAKGQPREPQVYTLPPSRDELTKNQVSLTCLVKGFYPSDIAVEWESNGQPENNYKTTPPVLDSDGSFFLYSKLTVDKSRWQQGNVFSCSVMHEGLHNHYTQKSLSLSPGK

SEQ ID NO: 78 - protein, 240 aa, synthetic construct
MDMKLPVRLLVLMFWIPGFSSDVLMTQTPLSLPVSLGDQASISCRASQSIVHTNGNTYLEWYLQKPGQSPKLLIYKVSNRFSGVPDRFSGSGSGTDFILKISRVEAEDLGVYYCFQGSHVPPTFGGGTKLEVKRADAAPTVSIFPPSSEQLTSGGASVVCLLNNFYPREAKVQWKVDNALQSGNSQESVTEQDSKDSTYSLSSTLTLSKADYEKHKVYACEVTHQGLSSPVTKSFNRGEC

SEQ ID NO: 79 - protein, 5 aa, synthetic construct
XYYIH

SEQ ID NO: 80 - protein, 16 aa, synthetic construct
RIDPENXXTTYAPKFQ

SEQ ID NO: 81 - protein, 11 aa, synthetic construct
RXSQSIVHTNG

SEQ ID NO: 82 - protein, 13 aa, synthetic construct
SPASXSVSLGDRX

SEQ ID NO: 83 - protein, 13 aa, synthetic construct
SPASXSVSLGDRX

SEQ ID NO: 84 - DNA, 36 bp, synthetic construct
  source 1..36: mol_type = other DNA
gtggtggaattcaccatgatgaaaaaaccagttgct

SEQ ID NO: 85 - DNA, 36 bp, synthetic construct
  source 1..36: mol_type = other DNA
gaagggccctctagattttgaaataagtgaatgacc

SEQ ID NO: 86 - DNA, 36 bp, synthetic construct
  source 1..36: mol_type = other DNA
gatgttggtctacctgatggtcaaatgggaaattca

SEQ ID NO: 87 - DNA, 36 bp, synthetic construct
  source 1..36: mol_type = other DNA
aagaccactagcatttatcaatgtgtttggatactc

SEQ ID NO: 88 - DNA, 36 bp, synthetic construct
  source 1..36: mol_type = other DNA
aaaactcaacttagagctgctgaaactgaaaagtat

SEQ ID NO: 89 - DNA, 36 bp, synthetic construct
  source 1..36: mol_type = other DNA
tccatttttagctagatactcacctagagtgttggc

SEQ ID NO: 90 - DNA, 36 bp, synthetic construct
  source 1..36: mol_type = other DNA
gtattaaactttgcaaatcctgatatggtaggtcat

SEQ ID NO: 91 - DNA, 36 bp, synthetic construct
  source 1..36: mol_type = other DNA
tataaagtcaaacttatcttctcctagtttatctaa

SEQ ID NO: 92 - DNA, 36 bp, synthetic construct
  source 1..36: mol_type = other DNA
atggaagcggcggttaaggctgttgaaactgtagat

SEQ ID NO: 93 - DNA, 36 bp, synthetic construct
  source 1..36: mol_type = other DNA
gctgaccacggtaacgctgaatatatgttagaccca

SEQ ID NO: 94 - DNA, 36 bp, synthetic construct
  source 1..36: mol_type = other DNA
accaacctgccagttccatttattgtagttggtcaa

SEQ ID NO: 95 - DNA, 36 bp, synthetic construct
  source 1..36: mol_type = other DNA
aaactttctgacatcgcaccgactgttttagatatg

SEQ ID NO: 96 - DNA, 36 bp, synthetic construct
  source 1..36: mol_type = other DNA
gtggtggaattcaccatgttggtttctaaaaaacct

SEQ ID NO: 97 - DNA, 36 bp, synthetic construct
  source 1..36: mol_type = other DNA
gaagggccctctagattccacgatgaacagcggctt

SEQ ID NO: 98 - DNA, 36 bp, synthetic construct
  source 1..36: mol_type = other DNA
aatgctagtggtcttgaagtcggtctgcctgaccgt

SEQ ID NO: 99 - DNA, 36 bp, synthetic construct
  source 1..36: mol_type = other DNA
cagaccggaagcgtcgatcagaggtagaccaacatc

SEQ ID NO: 100 - DNA, 36 bp, synthetic construct
  source 1..36: mol_type = other DNA
ctagctaaaaatggaaaaactcagttgcgtatttcc

SEQ ID NO: 101 - DNA, 36 bp, synthetic construct
  source 1..36: mol_type = other DNA
gtcgtttttcgccatccactctctaagttgagtttt

SEQ ID NO: 102 - DNA, 36 bp, synthetic construct
  source 1..36: mol_type = other DNA
aagtttgactttataatctgtaactatccgaacggc

SEQ ID NO: 103 - DNA, 36 bp, synthetic construct
  source 1..36: mol_type = other DNA
aatggtgtcgtatttgccgcttgcaaagtttaatac

SEQ ID NO: 104 - DNA, 17 bp, synthetic construct
  source 1..17: mol_type = other DNA
sargtnmagctgsagtc

SEQ ID NO: 105 - DNA, 23 bp, synthetic construct
  source 1..23: mol_type = other DNA
sargtnmagctgsagsagtcwgg

SEQ ID NO: 106 - DNA, 21 bp, synthetic construct
  source 1..21: mol_type = other DNA
caggttactctgaaagwtstg

SEQ ID NO: 107 - DNA, 20 bp, synthetic construct
  source 1..20: mol_type = other DNA
gaggtccarctgcaacartc

SEQ ID NO: 108 - DNA, 20 bp, synthetic construct
  source 1..20: mol_type = other DNA
caggtccaactvcagcarcc

SEQ ID NO: 109 - DNA, 20 bp, synthetic construct
  source 1..20: mol_type = other DNA
gaggtgaasstggtggaatc

SEQ ID NO: 110 - DNA, 20 bp, synthetic construct
  source 1..20: mol_type = other DNA
gatgtgaacttggaagtgtc

SEQ ID NO: 111 - DNA, 22 bp, synthetic construct
  source 1..22: mol_type = other DNA
gatggtgggatttctcgcagac

SEQ ID NO: 112 - DNA, 32 bp, synthetic construct
  source 1..32: mol_type = other DNA
ggctgcagsttcagtggcagtggrtcwggrac

SEQ ID NO: 113 - DNA, 21 bp, synthetic construct
  source 1..21: mol_type = other DNA
aacgtgagggtgctgctcatg

SEQ ID NO: 114 - protein, 479 aa, Mus musculus
MKFSWVIFFLMAVVTGVNSEVQLQQSLAELVRPGASVKLSCTASGFNIKNTYMHWVKQRPEQDLEWIGRIDPANGYTKYAPKFQGKATITADTSSNAAYLQLSSLTSEDTAIYYCGRGYSNFDYWGQGTTLTVSSESARNPTIYPLTLPRALSSDPVIIGCLIHDYFPSGTMNVTWGKSGKDITTVNFPPALASGGGYTMSSQLTLPAVECPEGESVKCSVQHDSNAVQELDVKCSGPPPPCPPCPPSCHPSLSLQRPALEDLLLGSDASLTCTLNGLRNPEGAVFTWEPSTGKDAVQKKAVQNSCGCYSVSSVLPGCAERWNSGASFKCTVTHPESDTLTGTIAKITVNTFPPQVHLLPPPSEELALNELVSLTCLVRAFNPKEVLVRWLHGNEELSPESYLVFEPLKEPGEGATTYLVTSVLRVSAELWKQGDQYSCMVGHEALPMNFTQKTIDRLSGKPTNVSVSVIMSEGDGICY

SEQ ID NO: 115 - protein, 135 aa, Mus musculus
MKFSWVIFFLMAVVTGVNSEVQLQQSLAELVRPGASVKLSCTASGFNIKNTYMHWVKQRPEQDLEWIGRIDPANGYTKYAPKFQGKATITADTSSNAAYLQLSSLTSEDTAIYYCGRGYSNFDYWGQGTTLTVSS

SEQ ID NO: 116 - protein, 8 aa, Mus musculus
GFNIKNTY

SEQ ID NO: 117 - protein, 8 aa, Mus musculus
IDPANGYT

SEQ ID NO: 118 - protein, 9 aa, Mus musculus
GRGYSNFDY

SEQ ID NO: 119 - protein, 236 aa, Mus musculus
MDMRTPAQFLGILLLWFPGFKCDIKMTQSPSSMYASLGERVTITCKASQDINSYLSWFQQKPGKSPKTLTYRANRLVDGVPSKFSGSGSGQDYSLTISSLEYEDMGIYYCLQYDEFPLTFGAGTKLELKRADAAPTVSIFPPSSEQLTSGGASVVCFLNNFYPKDINVKWKIDGSERQNGVLNSWTDQDSKDSTYSMSSTLTLTKDEYERHNSYTCEATHKTSTSPIVKSFNRNEC

SEQ ID NO: 120 - protein, 129 aa, Mus musculus
MDMRTPAQFLGILLLWFPGFKCDIKMTQSPSSMYASLGERVTITCKASQDINSYLSWFQQKPGKSPKTLTYRANRLVDGVPSKFSGSGSGQDYSLTISSLEYEDMGIYYCLQYDEFPLTFGAGTKLELK

SEQ ID NO: 121 - protein, 6 aa, Mus musculus
QDINSY

SEQ ID NO: 122 - skipped

SEQ ID NO: 123 - protein, 9 aa, Mus musculus
LQYDEFPLT

SEQ ID NO: 124 - protein, 484 aa, Mus musculus
MGWSWIFLLFLSGTAGVLSEVQLQQSGPEVVEPGASVKIPCKASGYTFTDYNMDWVKQSHGKSLEWIGDINPNNGGTIYNQKFKGQATLTVDKSSSTAYMELRSLTSEDTAVYYCAKSGYYGSGRYFDVWGTGTTVTVSSESARNPTIYPLTLPRALSSDPVIIGCLIHDYFPSGTMNVTWGKSGKDITTVNFPPALASGGGYTMSSQLTLPAVECPEGESVKCSVQHDSNAVQELDVKCSGPPPPCPPCPPSCHPSLSLQRPALEDLLLGSDASLTCTLNGLRNPEGAVFTWEPSTGKDAVQKKAVQNSCGCYSVSSVLPGCAERWNSGASFKCTVTHPESDTLTGTIAKITVNTFPPQVHLLPPPSEELALNELVSLTCLVRAFNPKEVLVRWLHGNEELSPESYLVFEPLKEPGEGATTYLVTSVLRVSAELWKQGDQYSCMVGHEALPMNFTQKTIDRLSGKPTNVSVSVIMSEGDGICY

SEQ ID NO: 125 - protein, 140 aa, Mus musculus
MGWSWIFLLFLSGTAGVLSEVQLQQSGPEVVEPGASVKIPCKASGYTFTDYNMDWVKQSHGKSLEWIGDINPNNGGTIYNQKFKGQATLTVDKSSSTAYMELRSLTSEDTAVYYCAKSGYYGSGRYFDVWGTGTTVTVSS

SEQ ID NO: 126 - protein, 8 aa, Mus musculus
GYTFTDYN

SEQ ID NO: 127 - protein, 8 aa, Mus musculus
INPNNGGT

SEQ ID NO: 128 - protein, 14 aa, Mus musculus
AKSGYYGSGRYFDV

SEQ ID NO: 129 - protein, 234 aa, Mus musculus
MVSTPQFLVFLLFWIPASRGDILLTQSPVILSVSPGERVSFSCRASQSIGSSIHWYQQRTNGSPRLLIKYASESISGIPSRFSGSGSGTDFTLTINSVASEDIADYYCQQSKSWPWTFGGGTKLEIKRADAAPTVSIFPPSSEQLTSGGASVVCFLNNFYPKDINVKWKIDGSERQNGVLNSWTDQDSKDSTYSMSSTLTLTKDEYERHNSYTCEATHKTSTSPIVKSFNRNEC

SEQ ID NO: 130 - protein, 127 aa, Mus musculus
MVSTPQFLVFLLFWIPASRGDILLTQSPVILSVSPGERVSFSCRASQSIGSSIHWYQQRTNGSPRLLIKYASESISGIPSRFSGSGSGTDFTLTINSVASEDIADYYCQQSKSWPWTFGGGTKLEIK

SEQ ID NO: 131 - protein, 6 aa, Mus musculus
QSIGSS

SEQ ID NO: 132 - skipped

SEQ ID NO: 133 - protein, 9 aa, Mus musculus
QQSKSWPWT

SEQ ID NO: 134 - DNA, 1440 bp, Mus musculus
  source 1..1440: mol_type = genomic DNA
atgaaattcagctgggtcatcttcttcctgatggcagtggttacaggggtcaattcagaggttcagctgcagcagtctctggcagagcttgtgaggccaggggcctcagtcaagttgtcctgcacagcttctggcttcaacatcaaaaacacctatatgcactgggtgaagcagaggcctgaacaggacctggagtggattggaaggattgatcctgcgaatggttatactaaatatgccccgaagttccagggcaaggccactataactgcagacacatcctccaacgcagcctacctgcagctcagcagcctgacatctgaggacactgccatctattactgtggtagaggctatagtaactttgactattggggccaaggcaccactctcacagtctcctcagagtctgcgagaaatcccaccatctacccactgacactcccacgagctctgtcaagtgacccagtgataatcggctgcctgattcacgattacttcccttccggcacgatgaatgtgacctggggaaagagtgggaaggatataaccaccgtaaacttcccacctgccctggcctctgggggagggtacaccatgagcagccagttgaccctgccagctgtcgagtgcccagaaggagaatccgtgaaatgttccgtgcaacatgactctaacgccgtccaagaattggatgtgaagtgctctggtcctcctcctccttgtcctccttgtcctccttcctgccatcccagcctgtcactgcagcggccagctcttgaggacctgctcctgggttcagatgccagcctcacatgtactctgaatggcctgagaaatcctgagggagctgtcttcacctgggagccctccactgggaaggatgcagtgcagaagaaagctgtgcagaattcctgcggctgctacagtgtgtccagcgtcctgcctggctgtgctgagcgctggaacagtggcgcatcattcaagtgcacagttacccatcctgagtctgacaccttaactggcacaattgccaaaatcacagtgaacaccttcccaccccaggtccacctgctaccgccgccgtcggaggagctggccctgaatgagctcgtgtccctgacatgcctggtgcgagctttcaaccctaaagaagtgctggtgcgatggctgcatggaaatgaggagctgtccccagaaagctacctagtgtttgagcccctaaaggagccaggcgagggagccaccacctacctggtgacaagcgtgttgcgtgtatcagctgaactctggaaacagggtgaccagtactcctgcatggtgggccacgaggccttgcccatgaacttcacccagaagaccatcgaccgtctgtcgggtaaacccaccaatgtcagcgtgtctgtgatcatgtcagagggagatggcatctgctactga

SEQ ID NO: 135 - DNA, 711 bp, Mus musculus
  source 1..711: mol_type = genomic DNA
atggacatgaggacccctgctcagtttcttggaatcttgttgctctggtttccaggtttcaaatgtgacatcaagatgacccagtctccatcttccatgtatgcatctctaggagagagagtcactatcacttgcaaggcgagtcaggacataaatagttatttaagctggttccagcagaaaccagggaaatctcctaagaccctgacctatcgtgcaaacagattggtagatggggtcccatcaaaattcagtggcagtggatctgggcaagattattctctcaccatcagcagcctggagtatgaagatatgggaatttattattgtctacagtatgatgagtttccgctcacgttcggtgctgggaccaagctggagctgaaacgggctgatgctgcaccaactgtatccatcttcccaccatccagtgagcagttaacatctggaggtgcctcagtcgtgtgcttcttgaacaacttctaccccaaagacatcaatgtcaagtggaagattgatggcagtgaacgacaaaatggcgtcctgaacagttggactgatcaggacagcaaagacagcacctacagcatgagcagcaccctcacgttgaccaaggacgagtatgaacgacataacagctatacctgtgaggccactcacaagacatcaacttcacccattgtcaagagcttcaacaggaatgagtgttga

SEQ ID NO: 136 - DNA, 1455 bp, Mus musculus
  source 1..1455: mol_type = genomic DNA
atgggatggagctggatctttctcctcttcctgtcaggaactgcaggtgtcctctctgaggtccaactgcaacagtctggacctgaagtggtggagcctggggcttcagtgaagataccctgcaaggcttctggatacacattcactgactacaacatggactgggtgaaacagagccatggaaagagccttgagtggattggcgatattaatccgaacaatggtggtactatctacaaccagaagttcaagggccaggccacattgactgttgacaagtcctccagtacagcctacatggagctccgcagcctgacatctgaggacactgcagtctattactgtgcaaaatcgggctactacggtagtggccggtacttcgatgtctggggcacagggaccacggtcaccgtctcctcagagtctgcgagaaatcccaccatctacccactgacactcccacgagctctgtcaagtgacccagtgataatcggctgcctgattcacgattacttcccttccggcacgatgaatgtgacctggggaaagagtgggaaggatataaccaccgtaaacttcccacctgccctggcctctgggggagggtacaccatgagcagccagttgaccctgccagctgtcgagtgcccagaaggagaatccgtgaaatgttccgtgcaacatgactctaacgccgtccaagaattggatgtgaagtgctctggtcctcctcctccttgtcctccttgtcctccttcctgccatcccagcctgtcactgcagcggccagctcttgaggacctgctcctgggttcagatgccagcctcacatgtactctgaatggcctgagaaatcctgagggagctgtcttcacctgggagccctccactgggaaggatgcagtgcagaagaaagctgtgcagaattcctgcggctgctacagtgtgtccagcgtcctgcctggctgtgctgagcgctggaacagtggcgcatcattcaagtgcacagttacccatcctgagtctgacaccttaactggcacaattgccaaaatcacagtgaacaccttcccaccccaggtccacctgctaccgccgccgtcggaggagctggccctgaatgagctcgtgtccctgacatgcctggtgcgagctttcaaccctaaagaagtgctggtgcgatggctgcatggaaatgaggagctgtccccagaaagctacctagtgtttgagcccctaaaggagccaggcgagggagccaccacctacctggtgacaagcgtgttgcgtgtatcagctgaactctggaaacagggtgaccagtactcctgcatggtgggccacgaggccttgcccatgaacttcacccagaagaccatcgaccgtctgtcgggtaaacccaccaatgtcagcgtgtctgtgatcatgtcagagggagatggcatctgctactga

SEQ ID NO: 137 - DNA, 705 bp, Mus musculus
  source 1..705: mol_type = genomic DNA
atggtatccacacctcagttccttgtatttttgcttttctggattccagcctccagaggtgacatcttgctgactcagtctccagtcatcctgtctgtgagtccaggagaaagagtcagtttctcctgcagggccagtcagagcattggctcaagcatacactggtatcagcaaagaacaaatggttctccaaggcttctcataaaatatgcttctgagtctatttctgggatcccttccaggtttagtggcagtggatcagggacagattttactcttaccatcaacagtgtggcgtctgaagacattgcagattattactgtcaacaaagtaaaagctggccgtggacgttcggtggaggcaccaaactggaaatcaaacgggctgatgctgcaccaactgtatccatcttcccaccatccagtgagcagttaacatctggaggtgcctcagtcgtgtgcttcttgaacaacttctaccccaaagacatcaatgtcaagtggaagattgatggcagtgaacgacaaaatggcgtcctgaacagttggactgatcaggacagcaaagacagcacctacagcatgagcagcaccctcacgttgaccaaggacgagtatgaacgacataacagctatacctgtgaggccactcacaagacatcaacttcacccattgtcaagagcttcaacaggaatgagtgttga